European Patent Application EP 4 353 740 A1, published April 17, 2024. Title: CONSTRUCT FOR INDUCING SILENCING IN PLANTS AND METHOD FOR PROTECTING THEM AGAINST ANTHRACNOSE DISEASE. Applicant: UNIVERSIDADE DE ÉVORA. Application EP. The sequence listing filed with the application follows.

SEQUENCE LISTING (3 sequences)

SEQ ID NO: 1 - DNA, 3678 bp, Olive mild mosaic virus
  source 1..3678: mol_type = genomic DNA
agtatacataccaagtatacggaataggtgtgaacccttgctcagctaaagaggataaaatggagctcactaaccactgcaagcaaactgctgctgaaggatttgtaagctttctgaactggctttgtaacccatggagacgacaacgaacagtcaacgctgctgttaagttccaacaggctctcctctcaatagaggatactgaacacttcgaggacatcaacgaatgcctcgaggagtctgctggagcccaatcacagcgaactaaggttgtcgccgaaggggcatattctcccgtcaaaaccaatcgtacccgccgagtccgcaagcagaagaaggccaagtttgtcaagtacttggtcaatgaggctcgtgccgagtttggtctacccaaagccactgaggccaatcgacttatggtacaacacttcttgctcagaacgtgtaaggaatggggtgtggtcacctcccaatgtcataacaacgttgcacttgcgttaaacctagtgttcatcccaactgaagatgacctgctgtcccgagcactgatgaacacttacgccacgcgagctgctgtgaatggaatgaccaacacccaaggggaggggtggtggaacaaccgacttgggattggatcccaggttggactggccttccgggccaaataggggtgcctagagaggaggccagggttctccacgtccgtttcgcgtggagagcaccctgatctggtggtcaaaccatcaggacaccccgagaaacagcgccagttgctgcgctatagtggaattggcggccatttactaattggcatccacaacaactctctctccaatttgcgccggggcttaatggaaagagtattctacgtcgagggacccaatgggctccaagacgccccgaaacccgacaagggagccttcaactcccttgctaagttcagagatctctatacaaagaatagctggcgtcattcccctgtaaccaatgagcaatttttgatgaattactcgggcaggaagctaactatttacaaggatgcggtcgacagtttgtcgcgtcaaccgcttagcctaagagatgctcggctgaagacattcgttaaggcggaaaaattgaatctgagtaagaaaccagatccagcaccgagggtcattcagcctcggtcgccccgctataacgtatgtttgggtcgttatcttcgtcactatgaacatcacgcgtttaaaaccattgctaaatgctttggggaaatcacggtctttaaaggattcactctcgagcaacaaggtgaaatcatgcactccaagtggaagaaatatgttaatcccgttgcggtcggtctcgatgccagtcgattcgatcaacacgtgtctagggaagcacttgagtacgagcatgaattttatttgagagattatcctaatgataaacagctaaaatggttgcttaagcaacaattgagtaatgtaggcacagcattcgctagcgacggaatcataaagtacaagaaagagggatgtagaatgagtggggacatgaacacaagtttgggaaactgcatattgatgtgcgccatggtctttgggctaaaagaacacttaggaatgaaattgtcattggctaacaatggggatgactgcgtcattgtctgtgagaaagcggatttattgaaattgacgagcagcatcgaaccatatttcagacagttcggattcaaaatggaagtggaaaagcctgtagacatctttgagcgcattgaattttgccaaacccaacctgtgttcgatggctcccaatacattatggttaggaaaccctccgttgtaacttccaaagatgtcactagcttaataccgtgccaaacacaatctcaatacgcagaatggctgcaagctgttggtgagtgcggtatgagcataaatggtggaatacctgtcatgcagaatttctacaccatgttgcaaactggcgtaaagcgcacaaaattcaccaagaccggcgagttccaggcgaatgggctagggtatcactctcgatttatgaacagggtggcccgaactccttcgcctgagacccgtttatccttttacttagcgtttggtatcacaccagacctccaggaagcattggaggtcttctatgataccagtacgcttgaattggatgatgtgatcccgactgatacctaccaagtgtcaggagagcatttaatcaatggattaccaaactgatatcaccgaagataacgtgagcataagcggtcgggccaggaggggcactggggacaagaaacacaatggttcgggaatgtctggcgtaaagcgtcatgcggtgagtgaaacagctcagaaatcgcagcaaggtactggcaatggcacaatgaccaacatagctgaagaacagaccattaccgtgacatacaactttaacttttgagttatggctgtgtgtcgctgctgtgatacttcaccaggtattacattattcccttactttgcaattctcatcctcatccttgcaatactagttgttggaactccaaaccagcaatatcatcattctcctagcatttacgagtacaagactcaacacatttcgatcgcaaaatagacatttactataacaccaaaacatgcctaagagaggacgagttggactcgctgaatcttttcaaagaaagacgaagcaacagaaacgggcagagtacgaagctgtaaaacgtgagcagctcgaacgtgcattcgcaaacaattccaaggtagccaatcctagatcttctgggctaagcttccgaccgttggtggcaccaatcgccgggtccgttgtttacagcagacctcgcgtgccacagatccgcacgaaccaaatgtcaactattgtggtaaacactgaattggtagccaacatcactttggctgctgctggagcattcagtttcaccgcccagccattgataccatcatttggatcttggttggccaacatagctgacttgtactcaaaatggagatggattaggtgttcagtcatatacatacctaaatgtcccaccaccactcaaggtagtgtggttatggcgattgtgtatgatgcgcaggacaccgtacctacgacacgaacgcaggtatcacagtgttatcaatccatcacatttccaccgtacgccgggtacggtggcgcctctgcgctaaatagctacagctctggaggggaatcgctagtgtctacacttgacaccaatcgcgttgataagaagtggtacagcacaataggcaatgctgccttcactgctctcacatctatcgacaagaaccagttctgtccagccacagctctcattgctggggacggcggacctgtgccttccacagctgtgggcgatgtatttatgcgatatgagattgagttcatcgaacgaatcaaccctaccattaacgtttgagtgttagttgcttaaaccctaagggtagatatgtgggcggtaagcaagagggatcctgggaaacaggcttcgacgggttgggggtggtgccccgaccgacgcatcacttgctgatacaaccattagacacctaagggcgggtctagccaggtctccacgccatgatcaattggaaacgattgtgaggggggtagtggaacccataccagattgaggggcctttgccccacccc

SEQ ID NO: 2 - DNA, 550 bp, Colletotrichum acutatum
  source 1..550: mol_type = genomic DNA
gcagtcgcagccctcagcctcgcgacggacgacatcgagaacctggtcaacgagctcagctccctcagtgtagtgacccttggcccagttgttgccggcaccggactggccaaagacgaagttgtcggggcggaaaagctggccaaagggaccggcacggacggcgtccatggtaccgggctccaagtcgacgaggacggcgcggggaacgtacttgttgccggaggcctggttgggtgagaaggtcagcattcgtcaataggattgcctgcacactggggggctaggataacaaacttcgttgaagtagacgctcatgcgctcgagctggagctcggaagtgccgttgtacctatggtatgattagctgctgggtccacggggaagccacactggaggacgagtgacatacacgccattgctgtcgagaccgtgctcgccagagatgttttgcctgtaccaaggtcagtacgagatcgtgtcaaatgtcggaatcgccgcgtcgctggcggttggctacgcaccagaaggcagcaccaatctggttacc

SEQ ID NO: 3 - DNA, 4228 bp, synthetic construct
  source 1..4228: mol_type = other DNA
agtatacataccaagtatacggaataggtgtgaacccttgctcagctaaagaggataaaatggagctcactaaccactgcaagcaaactgctgctgaaggatttgtaagctttctgaactggctttgtaacccatggagacgacaacgaacagtcaacgctgctgttaagttccaacaggctctcctctcaatagaggatactgaacacttcgaggacatcaacgaatgcctcgaggagtctgctggagcccaatcacagcgaactaaggttgtcgccgaaggggcatattctcccgtcaaaaccaatcgtacccgccgagtccgcaagcagaagaaggccaagtttgtcaagtacttggtcaatgaggctcgtgccgagtttggtctacccaaagccactgaggccaatcgacttatggtacaacacttcttgctcagaacgtgtaaggaatggggtgtggtcacctcccaatgtcataacaacgttgcacttgcgttaaacctagtgttcatcccaactgaagatgacctgctgtcccgagcactgatgaacacttacgccacgcgagctgctgtgaatggaatgaccaacacccaaggggaggggtggtggaacaaccgacttgggattggatcccaggttggactggccttccgggccaaataggggtgcctagagaggaggccagggttctccacgtccgtttcgcgtggagagcaccctgatctggtggtcaaaccatcaggacaccccgagaaacagcgccagttgctgcgctatagtggaattggcggccatttactaattggcatccacaacaactctctctccaatttgcgccggggcttaatggaaagagtattctacgtcgagggacccaatgggctccaagacgccccgaaacccgacaagggagccttcaactcccttgctaagttcagagatctctatacaaagaatagctggcgtcattcccctgtaaccaatgagcaatttttgatgaattactcgggcaggaagctaactatttacaaggatgcggtcgacagtttgtcgcgtcaaccgcttagcctaagagatgctcggctgaagacattcgttaaggcggaaaaattgaatctgagtaagaaaccagatccagcaccgagggtcattcagcctcggtcgccccgctataacgtatgtttgggtcgttatcttcgtcactatgaacatcacgcgtttaaaaccattgctaaatgctttggggaaatcacggtctttaaaggattcactctcgagcaacaaggtgaaatcatgcactccaagtggaagaaatatgttaatcccgttgcggtcggtctcgatgccagtcgattcgatcaacacgtgtctagggaagcacttgagtacgagcatgaattttatttgagagattatcctaatgataaacagctaaaatggttgcttaagcaacaattgagtaatgtaggcacagcattcgctagcgacggaatcataaagtacaagaaagagggatgtagaatgagtggggacatgaacacaagtttgggaaactgcatattgatgtgcgccatggtctttgggctaaaagaacacttaggaatgaaattgtcattggctaacaatggggatgactgcgtcattgtctgtgagaaagcggatttattgaaattgacgagcagcatcgaaccatatttcagacagttcggattcaaaatggaagtggaaaagcctgtagacatctttgagcgcattgaattttgccaaacccaacctgtgttcgatggctcccaatacattatggttaggaaaccctccgttgtaacttccaaagatgtcactagcttaataccgtgccaaacacaatctcaatacgcagaatggctgcaagctgttggtgagtgcggtatgagcataaatggtggaatacctgtcatgcagaatttctacaccatgttgcaaactggcgtaaagcgcacaaaattcaccaagaccggcgagttccaggcgaatgggctagggtatcactctcgatttatgaacagggtggcccgaactccttcgcctgagacccgtttatccttttacttagcgtttggtatcacaccagacctccaggaagcattggaggtcttctatgataccagtacgcttgaattggatgatgtgatcccgactgatacctaccaagtgtcaggagagcatttaatcaatggattaccaaactgatatcaccgaagataacgtgagcataagcggtcgggccaggaggggcactggggacaagaaacacaatggttcgggaatgtctggcgtaaagcgtcatgcggtgagtgaaacagctcagaaatcgcagcaaggtactggcaatggcacaatgaccaacatagctgaagaacagaccattaccgtgacatacaactttaacttttgagttatggctgtgtgtcgctgctgtgatacttcaccaggtattacattattcccttactttgcaattctcatcctcatccttgcaatactagttgttggaactccaaaccagcaatatcatcattctcctagcatttacgagtacaagactcaacacatttcgatcgcaaaatagacatttactataacaccaaaacatgcctaagagaggacgagttggactcgctgaatcttttcaaagaaagacgaagcaacagaaacgggcagagtacgaagctgtaaaacgtgagcagctcgaacgtgcattcgcaaacaattccaaggtagccaatcctagatcttctgggctaagcttccgaccgttggtggcaccaatcgccgggtccgttgtttacagcagacctcgcgtgccacagatccgcacgaaccaaatgtcaactattgtggtaaacactgaattggtagccaacatcactttggctgctgctggagcattcagtttcaccgcccagccattgataccatcatttggatcttggttggccaacatagctgacttgtactcaaaatggagatggattaggtgttcagtcatatacatacctaaatgtcccaccaccactcaaggtagtgtggttatggcgattgtgtatgatgcgcaggacaccgtacctacgacacgaacgcaggtatcacagtgttatcaatccatcacatttccaccgtacgccgggtacggtggcgcctctgcgctaaatagctacagctctggaggggaatcgctagtgtctacacttgacaccaatcgcgttgataagaagtggtacagcacaataggcaatgctgccttcactgctctcacatctatcgacaagaaccagttctgtccagccacagctctcattgctggggacggcggacctgtgccttccacagctgtgggcgatgtatttatgcgatatgagattgagttcatcgaacgaatcaaccctaccattaacgtttgagtgttagttgcagtcgcagccctcagcctcgcgacggacgacatcgagaacctggtcaacgagctcagctccctcagtgtagtgacccttggcccagttgttgccggcaccggactggccaaagacgaagttgtcggggcggaaaagctggccaaagggaccggcacggacggcgtccatggtaccgggctccaagtcgacgaggacggcgcggggaacgtacttgttgccggaggcctggttgggtgagaaggtcagcattcgtcaataggattgcctgcacactggggggctaggataacaaacttcgttgaagtagacgctcatgcgctcgagctggagctcggaagtgccgttgtacctatggtatgattagctgctgggtccacggggaagccacactggaggacgagtgacatacacgccattgctgtcgagaccgtgctcgccagagatgttttgcctgtaccaaggtcagtacgagatcgtgtcaaatgtcggaatcgccgcgtcgctggcggttggctacgcaccagaaggcagcaccaatctggttaccgcttaaaccctaagggtagatatgtgggcggtaagcaagagggatcctgggaaacaggcttcgacgggttgggggtggtgccccgaccgacgcatcacttgctgatacaaccattagacacctaagggcgggtctagccaggtctccacgccatgatcaattggaaacgattgtgaggggggtagtggaacccataccagattgaggggcctttgccccacccc